European Patent Specification EP 3 757 134 B1, published March 6, 2024. Title: CHLORIDE SALT OF TAT-NR2B9c. Applicant: NONO INC. GARMAN, JONATHAN DAVID. The sequence listing filed with the application follows.

SEQUENCE LISTING (73 sequences)

SEQ ID NO: 1 - protein, 10 aa, Artificial Sequence
  Synthesized
GRKKRRQRRR

SEQ ID NO: 2 - protein, 11 aa, Artificial Sequence
  Synthesized
YGRKKRRQRRR

SEQ ID NO: 3 - protein, 11 aa, Artificial Sequence
  Synthesized
FGRKKRRQRRR

SEQ ID NO: 4 - protein, 12 aa, Artificial Sequence
  Synthesized
GRKKRRQRRRPQ

SEQ ID NO: 5 - protein, 9 aa, Artificial Sequence
  Synthesized
KLSSIESDV

SEQ ID NO: 6 - protein, 20 aa, Artificial Sequence
  Synthesized
YGRKKRRQRRRKLSSIESDV

SEQ ID NO: 7 - protein, 20 aa, Artificial Sequence
  Synthesized
YGRKKRRQRRRKLSSIETDV

SEQ ID NO: 8 - protein, 12 aa, Artificial Sequence
  Synthesized
  VARIANT 1: Xaa = Blank or any amino acid
XFGRKKRRQRRR

SEQ ID NO: 9 - protein, 14 aa, Artificial Sequence
  Synthesized
RLSGMNEVLSFRWL

SEQ ID NO: 10 - protein, 9 aa, Artificial Sequence
  Synthesized
RRRQRRKKR

SEQ ID NO: 11 - protein, 20 aa, Artificial Sequence
  Synthesized
FNGSSNGHVYEKLSSIESDV

SEQ ID NO: 12 - protein, 4 aa, Artificial Sequence
  Synthesized
ESDV

SEQ ID NO: 13 - protein, 20 aa, Artificial Sequence
  Synthesized
HPTDITGPLNLSDPSVSTVV

SEQ ID NO: 14 - protein, 20 aa, Artificial Sequence
  Synthesized
RRAIEREEGQLQLCSRHRES

SEQ ID NO: 15 - protein, 20 aa, Artificial Sequence
  Synthesized
TQGFPGPCTWRRISSLESEV

SEQ ID NO: 16 - protein, 20 aa, Artificial Sequence
  Synthesized
AVSRKTELEEYQRTSRTCES

SEQ ID NO: 17 - protein, 20 aa, Artificial Sequence
  Synthesized
LNSCSNRRVYKKMPSIESDV

SEQ ID NO: 18 - protein, 20 aa, Artificial Sequence
  Synthesized
GGDLGTRRGSAHFSSLESEV

SEQ ID NO: 19 - protein, 20 aa, Artificial Sequence
  Synthesized
QPTPTLGLNLGNDPDRGTSI

SEQ ID NO: 20 - protein, 20 aa, Artificial Sequence
  Synthesized
MQSIPCMSHSSGMPLGATGL

SEQ ID NO: 21 - protein, 20 aa, Artificial Sequence
  Synthesized
QNFATYKEGYNVYGIESVKI

SEQ ID NO: 22 - protein, 20 aa, Artificial Sequence
  Synthesized
QNYATYREGYNVYGTESVKI

SEQ ID NO: 23 - protein, 20 aa, Artificial Sequence
  Synthesized
HTGTAIRQSSGLAVIASDLP

SEQ ID NO: 24 - protein, 20 aa, Artificial Sequence
  Synthesized
SFTSILTCHQRRTQRKETVA

SEQ ID NO: 25 - protein, 20 aa, Artificial Sequence
  Synthesized
EVINMHTFNDRRLPGKETMA

SEQ ID NO: 26 - protein, 5 aa, Artificial Sequence
  Synthesized
IETAV

SEQ ID NO: 27 - protein, 4 aa, Artificial Sequence
  Synthesized
STVV

SEQ ID NO: 28 - protein, 4 aa, Artificial Sequence
  Synthesized
HRES

SEQ ID NO: 29 - protein, 4 aa, Artificial Sequence
  Synthesized
ESEV

SEQ ID NO: 30 - protein, 4 aa, Artificial Sequence
  Synthesized
TCES

SEQ ID NO: 31 - protein, 4 aa, Artificial Sequence
  Synthesized
GTSI

SEQ ID NO: 32 - protein, 4 aa, Artificial Sequence
  Synthesized
ATGL

SEQ ID NO: 33 - protein, 4 aa, Artificial Sequence
  Synthesized
SVKI

SEQ ID NO: 34 - protein, 4 aa, Artificial Sequence
  Synthesized
SDLP

SEQ ID NO: 35 - protein, 4 aa, Artificial Sequence
  Synthesized
ETVA

SEQ ID NO: 36 - protein, 4 aa, Artificial Sequence
  Synthesized
ETMA

SEQ ID NO: 37 - protein, 20 aa, Artificial Sequence
  Synthesized
RRRQRRKKRGYKLSSIETDV

SEQ ID NO: 38 - protein, 4 aa, Artificial Sequence
  Synthesized
  VARIANT 1: Xaa = E, D, N, or Q
  VARIANT 2: Xaa = S or T
  VARIANT 3: Xaa = D, E, Q, or N
  VARIANT 4: Xaa = V or L
XXXX

SEQ ID NO: 39 - protein, 4 aa, Artificial Sequence
  Synthesized
ETDV

SEQ ID NO: 40 - protein, 4 aa, Artificial Sequence
  Synthesized
ETEV

SEQ ID NO: 41 - protein, 4 aa, Artificial Sequence
  Synthesized
DTDV

SEQ ID NO: 42 - protein, 4 aa, Artificial Sequence
  Synthesized
DTEV

SEQ ID NO: 43 - protein, 9 aa, Artificial Sequence
  Synthesized
KLSSIETDV

SEQ ID NO: 44 - protein, 5 aa, Artificial Sequence
  Synthesized
GSSSS

SEQ ID NO: 45 - protein, 5 aa, Artificial Sequence
  Synthesized
TGEKP

SEQ ID NO: 46 - protein, 8 aa, Artificial Sequence
  Synthesized
GGRRGGGS

SEQ ID NO: 47 - protein, 9 aa, Artificial Sequence
  Synthesized
LRQRDGERP

SEQ ID NO: 48 - protein, 13 aa, Artificial Sequence
  Synthesized
YGRKKRRQRRRPQ

SEQ ID NO: 49 - protein, 11 aa, Artificial Sequence
  Synthesized
  VARIANT 1: Xaa = Blank or an amino acid that is not Y
XGRKKRRQRRR

SEQ ID NO: 50 - protein, 11 aa, Artificial Sequence
  Synthesized
  VARIANT 1: Xaa = Blank or any amino acid
XGKKKKKQKKK

SEQ ID NO: 51 - protein, 10 aa, Artificial Sequence
  Synthesized
  VARIANT 1: Xaa = Blank or any amino acid
XRKKRRQRRR

SEQ ID NO: 52 - protein, 11 aa, Artificial Sequence
  Synthesized
  VARIANT 1: Xaa = Blank or any amino acid
XGAKKRRQRRR

SEQ ID NO: 53 - protein, 10 aa, Artificial Sequence
  Synthesized
  VARIANT 1: Xaa = Blank or any amino acid
XAKKRRQRRR

SEQ ID NO: 54 - protein, 11 aa, Artificial Sequence
  Synthesized
  VARIANT 1: Xaa = Blank or any amino acid
XGRKARRQRRR

SEQ ID NO: 55 - protein, 10 aa, Artificial Sequence
  Synthesized
  VARIANT 1: Xaa = Blank or any amino acid
XRKARRQRRR

SEQ ID NO: 56 - protein, 11 aa, Artificial Sequence
  Synthesized
  VARIANT 1: Xaa = Blank or any amino acid
XGRKKARQRRR

SEQ ID NO: 57 - protein, 10 aa, Artificial Sequence
  Synthesized
  VARIANT 1: Xaa = Blank or any amino acid
XRKKARQRRR

SEQ ID NO: 58 - protein, 11 aa, Artificial Sequence
  Synthesized
  VARIANT 1: Xaa = Blank or any amino acid
XGRKKRRQARR

SEQ ID NO: 59 - protein, 10 aa, Artificial Sequence
  Synthesized
  VARIANT 1: Xaa = Blank or any amino acid
XRKKRRQARR

SEQ ID NO: 60 - protein, 11 aa, Artificial Sequence
  Synthesized
  VARIANT 1: Xaa = Blank or any amino acid
XGRKKRRQRAR

SEQ ID NO: 61 - protein, 10 aa, Artificial Sequence
  Synthesized
  VARIANT 1: Xaa = Blank or any amino acid
XRKKRRQRAR

SEQ ID NO: 62 - protein, 12 aa, Artificial Sequence
  Synthesized
  VARIANT 1: Xaa = Blank or any amino acid
XRRPRRPRRPRR

SEQ ID NO: 63 - protein, 12 aa, Artificial Sequence
  Synthesized
  VARIANT 1: Xaa = Blank or any amino acid
XRRARRARRARR

SEQ ID NO: 64 - protein, 11 aa, Artificial Sequence
  Synthesized
  VARIANT 1: Xaa = Blank or any amino acid
XRRRARRRARR

SEQ ID NO: 65 - protein, 11 aa, Artificial Sequence
  Synthesized
  VARIANT 1: Xaa = Blank or any amino acid
XRRRPRRRPRR

SEQ ID NO: 66 - protein, 9 aa, Artificial Sequence
  Synthesized
  VARIANT 1: Xaa = Blank or any amino acid
XRRPRRPRR

SEQ ID NO: 67 - protein, 9 aa, Artificial Sequence
  Synthesized
  VARIANT 1: Xaa = Blank or any amino acid
XRRARRARR

SEQ ID NO: 68 - protein, 4 aa, Artificial Sequence
  Synthesized
  VARIANT 1: Xaa = E, Q, A, or an analog therof
  VARIANT 2: Xaa = T or S
  VARIANT 3: Xaa = A, Q, D, N, N-Me-A, N-Me-Q, N-Me-D, N-Me-N, or an analogue thereof
XXXV

SEQ ID NO: 69 - protein, 22 aa, Artificial Sequence
  Synthesized
VDSEISSLKRRRQRRKKRGYIN

SEQ ID NO: 70 - protein, 20 aa, Artificial Sequence
  Synthesized
RRRQRRKKRGYKLSSIESDV

SEQ ID NO: 71 - protein, 5 aa, Artificial Sequence
  Synthesized
IESDV

SEQ ID NO: 72 - protein, 11 aa, Artificial Sequence
  Synthesized
GRKKRRQRRRP

SEQ ID NO: 73 - protein, 5 aa, Artificial Sequence
  Synthesized
IETDV